European Patent Application EP 4 310 189 A1, published January 24, 2024. Title: Mutant of Corynebacterium glutamicum with enhanced L-citrulline productivity and method for preparing L-citrulline using the same. Applicant: DAESANG CORPORATION. The sequence listing filed with the application follows.

SEQUENCE LISTING (10 sequences)

SEQ ID NO: 1 - DNA, 1386 bp, Artificial Sequence
  NCgl2657 gene
atgtctgacacaccgacctcagctctgatcaccacggtcaaccgcagcttcgatggattcgatttggaagaagtagcagcagaccttggagttcggctcacctacctgcccgacgaagaactagaagtatccaaagttctcgcggcggacctcctcgctgaggggccagctctcatcatcggtgtaggaaacacgtttttcgacgcccaggtcgccgctgccctcggcgtcccagtgctactgctggtagacaagcaaggcaagcacgttgctcttgctcgcacccaggtaaacaatgccggcgcagttgttgcagcagcatttaccgctgaacaagagccaatgccggataagctgcgcaaggctgtgcgcaaccacagcaacctcgaaccagtcatgagcgccgaactctttgaaaactggctgctcaagcgcgcacgcgcagagcactcccacattgtgctgccagaaggtgacgacgaccgcatcttgatggctgcccaccagctgcttgatcaagacatctgtgacatcacgatcctgggcgatccagtaaagatcaaggagcgcgctaccgaacttggcctgcaccttaacactgcatacctggtcaatccgctgacagatcctcgcctggaggaattcgccgaacaattcgcggagctgcgcaagtcaaagagcgtcactatcgatgaagcccgcgaaatcatgaaggatatttcctacttcggcaccatgatggtccacaacggcgacgccgacggaatggtatccggtgcagcaaacaccaccgcacacaccattaagccaagcttccagatcatcaaaactgttccagaagcatccgtcgtttcttccatcttcctcatggtgctgcgcgggcgactgtgggcattcggcgactgtgctgttaacccgaacccaactgctgaacagcttggtgaaatcgccgttgtgtcagcaaaaactgcagcacaatttggcattgatcctcgcgtagccatcttgtcctactccactggcaactccggcggaggctcagatgtggatcgcgccatcgacgctcttgcagaagcacgccgacttaacccagaactatgcgtcgatggaccacttcagttcgacgccgccgtcgacccgggtgtggcgcgcaagaagatgccagactctgacgtcgctggccaggcaaatgtgtttatcttccctgacctggaagccggaaacatcggctacaaaactgcacaacgcaccggtcacgccctggcagttggtccgattctgcagggcctaaacaaaccagtcaacgacctttcccgtggcgcaacagtccctgacatcgtcaacacagtagccatcacagcaattcaggcaggaggacgcagctaa

SEQ ID NO: 2 - DNA, 1386 bp, Artificial Sequence
  NCgl2657 gene - substituted ATG with TTG
ttgtctgacacaccgacctcagctctgatcaccacggtcaaccgcagcttcgatggattcgatttggaagaagtagcagcagaccttggagttcggctcacctacctgcccgacgaagaactagaagtatccaaagttctcgcggcggacctcctcgctgaggggccagctctcatcatcggtgtaggaaacacgtttttcgacgcccaggtcgccgctgccctcggcgtcccagtgctactgctggtagacaagcaaggcaagcacgttgctcttgctcgcacccaggtaaacaatgccggcgcagttgttgcagcagcatttaccgctgaacaagagccaatgccggataagctgcgcaaggctgtgcgcaaccacagcaacctcgaaccagtcatgagcgccgaactctttgaaaactggctgctcaagcgcgcacgcgcagagcactcccacattgtgctgccagaaggtgacgacgaccgcatcttgatggctgcccaccagctgcttgatcaagacatctgtgacatcacgatcctgggcgatccagtaaagatcaaggagcgcgctaccgaacttggcctgcaccttaacactgcatacctggtcaatccgctgacagatcctcgcctggaggaattcgccgaacaattcgcggagctgcgcaagtcaaagagcgtcactatcgatgaagcccgcgaaatcatgaaggatatttcctacttcggcaccatgatggtccacaacggcgacgccgacggaatggtatccggtgcagcaaacaccaccgcacacaccattaagccaagcttccagatcatcaaaactgttccagaagcatccgtcgtttcttccatcttcctcatggtgctgcgcgggcgactgtgggcattcggcgactgtgctgttaacccgaacccaactgctgaacagcttggtgaaatcgccgttgtgtcagcaaaaactgcagcacaatttggcattgatcctcgcgtagccatcttgtcctactccactggcaactccggcggaggctcagatgtggatcgcgccatcgacgctcttgcagaagcacgccgacttaacccagaactatgcgtcgatggaccacttcagttcgacgccgccgtcgacccgggtgtggcgcgcaagaagatgccagactctgacgtcgctggccaggcaaatgtgtttatcttccctgacctggaagccggaaacatcggctacaaaactgcacaacgcaccggtcacgccctggcagttggtccgattctgcagggcctaaacaaaccagtcaacgacctttcccgtggcgcaacagtccctgacatcgtcaacacagtagccatcacagcaattcaggcaggaggacgcagctaa

SEQ ID NO: 3 - DNA, 40 bp, Artificial Sequence
  Primer 1
ctatgaccatgattacgccacagtggagaacacgatcgcg

SEQ ID NO: 4 - DNA, 40 bp, Artificial Sequence
  Primer 2
gaggtcggtgtgtcagacaaacatcgcctttctaatttca

SEQ ID NO: 5 - DNA, 40 bp, Artificial Sequence
  Primer 3
tgaaattagaaaggcgatgtttgtctgacacaccgacctc

SEQ ID NO: 6 - DNA, 40 bp, Artificial Sequence
  Primer 4
gctcggtacccggggatcctcggcgtcgccgttgtggacc

SEQ ID NO: 7 - DNA, 40 bp, Artificial Sequence; identical to SEQ ID NO: 3
  Primer 5

SEQ ID NO: 8 - DNA, 40 bp, Artificial Sequence
  Primer 6
caaaacaagtgccaatgccaacatcgcctttctaatttca

SEQ ID NO: 9 - DNA, 40 bp, Artificial Sequence
  Primer 7
tgaaattagaaaggcgatgttggcattggcacttgttttg

SEQ ID NO: 10 - DNA, 40 bp, Artificial Sequence
  Primer 8
gctcggtacccggggatcctatcgatgctcatgccagcgg